European Patent Application EP 4 745 157 A1, published May 20, 2026. Title: 신규 TM4SF5-특이적 항체. Applicant: 한국생명공학연구원. The sequence listing filed with the application follows.

SEQUENCE LISTING (71 sequences)

SEQ ID NO: 1 - protein, 114 aa, synthetic construct
  source 1..114: note = Ab27-hz9_VH
QVQLVQSGAEVKKPGASVKVSCKASGYTFTDYEMHWVRQAPGQGLEWMGAIDPETGGTAYNQKFKGRVTMTADKSISTAYMELSRLRSDDTAVYYCARPYLGYWGQGTLVTVSS

SEQ ID NO: 2 - protein, 444 aa, synthetic construct
  source 1..444: note = Ab27-hz9_Heavy chain
QVQLVQSGAEVKKPGASVKVSCKASGYTFTDYEMHWVRQAPGQGLEWMGAIDPETGGTAYNQKFKGRVTMTADKSISTAYMELSRLRSDDTAVYYCARPYLGYWGQGTLVTVSSASTKGPSVFPLAPSSKSTSGGTAALGCLVKDYFPEPVTVSWNSGALTSGVHTFPAVLQSSGLYSLSSVVTVPSSSLGTQTYICNVNHKPSNTKVDKKVEPKSCDKTHTCPPCPAPELLGGPSVFLFPPKPKDTLMISRTPEVTCVVVDVSHEDPEVKFNWYVDGVEVHNAKTKPREEQYNSTYRVVSVLTVLHQDWLNGKEYKCKVSNKALPAPIEKTISKAKGQPREPQVYTLPPSRDELTKNQVSLTCLVKGFYPSDIAVEWESNGQPENNYKTTPPVLDSDGSFFLYSKLTVDKSRWQQGNVFSCSVMHEALHNHYTQKSLSLSPGK

SEQ ID NO: 3 - protein, 5 aa, synthetic construct
  source 1..5: note = Ab27-hz9_HCDR1_Kabat
DYEMH

SEQ ID NO: 4 - protein, 17 aa, synthetic construct
  source 1..17: note = Ab27-hz9_HCDR2_Kabat
AIDPETGGTAYNQKFKG

SEQ ID NO: 5 - protein, 5 aa, synthetic construct
  source 1..5: note = Ab27-hz9_HCDR3_Kabat
PYLGY

SEQ ID NO: 6 - protein, 7 aa, synthetic construct
  source 1..7: note = Ab27-hz9_HCDR1_Chothia
GYTFTDY

SEQ ID NO: 7 - protein, 6 aa, synthetic construct
  source 1..6: note = Ab27-hz9_HCDR2_Chothia
DPETGG

SEQ ID NO: 8 - protein, 5 aa, synthetic construct
  source 1..5: note = Ab27-hz9_HCDR3_Chothia
PYLGY

SEQ ID NO: 9 - protein, 112 aa, synthetic construct
  source 1..112: note = VL
EIVLTQSPGTLSLSPGERATLSCRSSQSLVHSNGNTYLHWYQQKPGQAPRLLIYKVSNRFSGIPDRFSGSGSGTDFTLTISRLEPEDFAVYYCFQGSHIPLTFGQGTKVEIK

SEQ ID NO: 10 - protein, 219 aa, synthetic construct
  source 1..219: note = Ab27-hz9_Light chain
EIVLTQSPGTLSLSPGERATLSCRSSQSLVHSNGNTYLHWYQQKPGQAPRLLIYKVSNRFSGIPDRFSGSGSGTDFTLTISRLEPEDFAVYYCFQGSHIPLTFGQGTKVEIKRTVAAPSVFIFPPSDEQLKSGTASVVCLLNNFYPREAKVQWKVDNALQSGNSQESVTEQDSKDSTYSLSSTLTLSKADYEKHKVYACEVTHQGLSSPVTKSFNRGEC

SEQ ID NO: 11 - protein, 16 aa, synthetic construct
  source 1..16: note = LCDR1
RSSQSLVHSNGNTYLH

SEQ ID NO: 12 - protein, 7 aa, synthetic construct
  source 1..7: note = LCDR2
KVSNRFS

SEQ ID NO: 13 - protein, 9 aa, synthetic construct
  source 1..9: note = LCDR3
FQGSHIPLT

SEQ ID NO: 14 - protein, 114 aa, synthetic construct
  source 1..114: note = S43_VH
QVQLVQSGAEVKKPGASVKVSCKASGYRFTDYEMHWVRQAPGQGLEWMGAIDPAFGGTAYNQKFKGRVTMTADKSISTAYMELSRLRSDDTAVYYCARPYLGYWGQGTLVTVSS

SEQ ID NO: 15 - protein, 444 aa, synthetic construct
  source 1..444: note = S43_heavy chain
QVQLVQSGAEVKKPGASVKVSCKASGYRFTDYEMHWVRQAPGQGLEWMGAIDPAFGGTAYNQKFKGRVTMTADKSISTAYMELSRLRSDDTAVYYCARPYLGYWGQGTLVTVSSASTKGPSVFPLAPSSKSTSGGTAALGCLVKDYFPEPVTVSWNSGALTSGVHTFPAVLQSSGLYSLSSVVTVPSSSLGTQTYICNVNHKPSNTKVDKKVEPKSCDKTHTCPPCPAPELLGGPSVFLFPPKPKDTLMISRTPEVTCVVVDVSHEDPEVKFNWYVDGVEVHNAKTKPREEQYNSTYRVVSVLTVLHQDWLNGKEYKCKVSNKALPAPIEKTISKAKGQPREPQVYTLPPSRDELTKNQVSLTCLVKGFYPSDIAVEWESNGQPENNYKTTPPVLDSDGSFFLYSKLTVDKSRWQQGNVFSCSVMHEALHNHYTQKSLSLSPGK

SEQ ID NO: 16 - protein, 5 aa, synthetic construct
  source 1..5: note = S43_HCDR1_Kabat
DYEMH

SEQ ID NO: 17 - protein, 17 aa, synthetic construct
  source 1..17: note = S43_HCDR2_Kabat
AIDPAFGGTAYNQKFKG

SEQ ID NO: 18 - protein, 5 aa, synthetic construct
  source 1..5: note = S43_HCDR3_Kabat
PYLGY

SEQ ID NO: 19 - protein, 7 aa, synthetic construct
  source 1..7: note = S43_HCDR1_Chothia
GYRFTDY

SEQ ID NO: 20 - protein, 6 aa, synthetic construct
  source 1..6: note = S43_HCDR2_Chothia
DPAFGG

SEQ ID NO: 21 - protein, 5 aa, synthetic construct
  source 1..5: note = S43_HCDR3_Chothia
PYLGY

SEQ ID NO: 22 - protein, 114 aa, synthetic construct
  source 1..114: note = 1-5_VH
QVQLVQSGAEVKKPGASVKVSCKASGYTFTDYEMHWVRQAPGQGLEWMGAIDPETGGTFVKRKFKGRVTMTADKSISTAYMELSRLRSDDTAVYYCARPYLGYWGQGTLVTVSS

SEQ ID NO: 23 - protein, 444 aa, synthetic construct
  source 1..444: note = 1-5_Heavy chain
QVQLVQSGAEVKKPGASVKVSCKASGYTFTDYEMHWVRQAPGQGLEWMGAIDPETGGTFVKRKFKGRVTMTADKSISTAYMELSRLRSDDTAVYYCARPYLGYWGQGTLVTVSSASTKGPSVFPLAPSSKSTSGGTAALGCLVKDYFPEPVTVSWNSGALTSGVHTFPAVLQSSGLYSLSSVVTVPSSSLGTQTYICNVNHKPSNTKVDKKVEPKSCDKTHTCPPCPAPELLGGPSVFLFPPKPKDTLMISRTPEVTCVVVDVSHEDPEVKFNWYVDGVEVHNAKTKPREEQYNSTYRVVSVLTVLHQDWLNGKEYKCKVSNKALPAPIEKTISKAKGQPREPQVYTLPPSRDELTKNQVSLTCLVKGFYPSDIAVEWESNGQPENNYKTTPPVLDSDGSFFLYSKLTVDKSRWQQGNVFSCSVMHEALHNHYTQKSLSLSPGK

SEQ ID NO: 24 - protein, 5 aa, synthetic construct
  source 1..5: note = 1-5_HCDR1_Kabat
DYEMH

SEQ ID NO: 25 - protein, 17 aa, synthetic construct
  source 1..17: note = 1-5_HCDR2_Kabat
AIDPETGGTFVKRKFKG

SEQ ID NO: 26 - protein, 5 aa, synthetic construct
  source 1..5: note = 1-5_HCDR3_Kabat
PYLGY

SEQ ID NO: 27 - protein, 7 aa, synthetic construct
  source 1..7: note = 1-5_HCDR1_Chothia
GYTFTDY

SEQ ID NO: 28 - protein, 6 aa, synthetic construct
  source 1..6: note = 1-5_HCDR2_Chothia
DPETGG

SEQ ID NO: 29 - protein, 5 aa, synthetic construct
  source 1..5: note = 1-5_HCDR3_Chothia
PYLGY

SEQ ID NO: 30 - protein, 114 aa, synthetic construct
  source 1..114: note = 2-1_VH
QVQLVQSGAEVKKPGASVKVSCKASGYTFTDYEMHWVRQAPGQGLEWMGAIDPETGGTFVVSKFKGRVTMTADKSISTAYMELSRLRSDDTAVYYCARPYLGYWGQGTLVTVSS

SEQ ID NO: 31 - protein, 444 aa, synthetic construct
  source 1..444: note = 2-1_Heavy chain
QVQLVQSGAEVKKPGASVKVSCKASGYTFTDYEMHWVRQAPGQGLEWMGAIDPETGGTFVVSKFKGRVTMTADKSISTAYMELSRLRSDDTAVYYCARPYLGYWGQGTLVTVSSASTKGPSVFPLAPSSKSTSGGTAALGCLVKDYFPEPVTVSWNSGALTSGVHTFPAVLQSSGLYSLSSVVTVPSSSLGTQTYICNVNHKPSNTKVDKKVEPKSCDKTHTCPPCPAPELLGGPSVFLFPPKPKDTLMISRTPEVTCVVVDVSHEDPEVKFNWYVDGVEVHNAKTKPREEQYNSTYRVVSVLTVLHQDWLNGKEYKCKVSNKALPAPIEKTISKAKGQPREPQVYTLPPSRDELTKNQVSLTCLVKGFYPSDIAVEWESNGQPENNYKTTPPVLDSDGSFFLYSKLTVDKSRWQQGNVFSCSVMHEALHNHYTQKSLSLSPGK

SEQ ID NO: 32 - protein, 5 aa, synthetic construct
  source 1..5: note = 2-1_HCDR1_Kabat
DYEMH

SEQ ID NO: 33 - protein, 17 aa, synthetic construct
  source 1..17: note = 2-1_HCDR2_Kabat
AIDPETGGTFVVSKFKG

SEQ ID NO: 34 - protein, 5 aa, synthetic construct
  source 1..5: note = 2-1_HCDR3_Kabat
PYLGY

SEQ ID NO: 35 - protein, 7 aa, synthetic construct
  source 1..7: note = 2-1_HCDR1_Chothia
GYTFTDY

SEQ ID NO: 36 - protein, 6 aa, synthetic construct
  source 1..6: note = 2-1_HCDR2_Chothia
DPETGG

SEQ ID NO: 37 - protein, 5 aa, synthetic construct
  source 1..5: note = 2-1_HCDR3_Chothia
PYLGY

SEQ ID NO: 38 - protein, 114 aa, synthetic construct
  source 1..114: note = E01_VH
EVQLVQSGADVKEPGASVKVSCKASGYTFTDYEMHWVRQAPGQGLEWMGAIDPETGGTAYNQKFKGWVTMTADKSISTAYMELSRLRSDDTAVYYCTRPYLGYWGQGTLVTVSS

SEQ ID NO: 39 - protein, 444 aa, synthetic construct
  source 1..444: note = E01_Heavy chain
EVQLVQSGADVKEPGASVKVSCKASGYTFTDYEMHWVRQAPGQGLEWMGAIDPETGGTAYNQKFKGWVTMTADKSISTAYMELSRLRSDDTAVYYCTRPYLGYWGQGTLVTVSSASTKGPSVFPLAPSSKSTSGGTAALGCLVKDYFPEPVTVSWNSGALTSGVHTFPAVLQSSGLYSLSSVVTVPSSSLGTQTYICNVNHKPSNTKVDKKVEPKSCDKTHTCPPCPAPELLGGPSVFLFPPKPKDTLMISRTPEVTCVVVDVSHEDPEVKFNWYVDGVEVHNAKTKPREEQYNSTYRVVSVLTVLHQDWLNGKEYKCKVSNKALPAPIEKTISKAKGQPREPQVYTLPPSRDELTKNQVSLTCLVKGFYPSDIAVEWESNGQPENNYKTTPPVLDSDGSFFLYSKLTVDKSRWQQGNVFSCSVMHEALHNHYTQKSLSLSPGK

SEQ ID NO: 40 - protein, 5 aa, synthetic construct
  source 1..5: note = E01_HCDR1_Kabat
DYEMH

SEQ ID NO: 41 - protein, 17 aa, synthetic construct
  source 1..17: note = E01_HCDR2_Kabat
AIDPETGGTAYNQKFKG

SEQ ID NO: 42 - protein, 5 aa, synthetic construct
  source 1..5: note = E01_HCDR3_Kabat
PYLGY

SEQ ID NO: 43 - protein, 7 aa, synthetic construct
  source 1..7: note = E01_HCDR1_Chothia
GYTFTDY

SEQ ID NO: 44 - protein, 6 aa, synthetic construct
  source 1..6: note = E01_HCDR2_Chothia
DPETGG

SEQ ID NO: 45 - protein, 5 aa, synthetic construct
  source 1..5: note = E01_HCDR3_Chothia
PYLGY

SEQ ID NO: 46 - protein, 112 aa, synthetic construct
  source 1..112: note = E01_VL
EIVLTQSPGMLSLSPGERATLSCRSSQSLVHRNGNTYLHWYQQKPGQAPRLLIYKVSNRFSGIPDRFSGSGSGTDFTLTISRLEPEDFAVYYCFQGSHIPLTFGQGTKVEIK

SEQ ID NO: 47 - protein, 219 aa, synthetic construct
  source 1..219: note = E01_Light chain
EIVLTQSPGMLSLSPGERATLSCRSSQSLVHRNGNTYLHWYQQKPGQAPRLLIYKVSNRFSGIPDRFSGSGSGTDFTLTISRLEPEDFAVYYCFQGSHIPLTFGQGTKVEIKRTVAAPSVFIFPPSDEQLKSGTASVVCLLNNFYPREAKVQWKVDNALQSGNSQESVTEQDSKDSTYSLSSTLTLSKADYEKHKVYACEVTHQGLSSPVTKSFNRGEC

SEQ ID NO: 48 - protein, 16 aa, synthetic construct
  source 1..16: note = E01_LCDR1
RSSQSLVHRNGNTYLH

SEQ ID NO: 49 - protein, 7 aa, synthetic construct
  source 1..7: note = E01_LCDR2
KVSNRFS

SEQ ID NO: 50 - protein, 9 aa, synthetic construct
  source 1..9: note = E01_LCDR3
FQGSHIPLT

SEQ ID NO: 51 - protein, 8 aa, synthetic construct
  source 1..8: note = Ab27-hz9_HCDR1_IMGT
GYTFTDYE

SEQ ID NO: 52 - protein, 8 aa, synthetic construct
  source 1..8: note = Ab27-hz9_HCDR2_IMGT
IDPETGGT

SEQ ID NO: 53 - protein, 7 aa, synthetic construct
  source 1..7: note = Ab27-hz9_HCDR3_IMGT
ARPYLGY

SEQ ID NO: 54 - protein, 11 aa, synthetic construct
  source 1..11: note = Ab27-hz9_LCDR1_IMGT
QSLVHSNGNTY

SEQ ID NO: 55 - skipped

SEQ ID NO: 56 - protein, 9 aa, synthetic construct
  source 1..9: note = Ab27-hz9_LCDR3_IMGT
FQGSHIPLT

SEQ ID NO: 57 - protein, 8 aa, synthetic construct
  source 1..8: note = S43_HCDR1_IMGT
GYRFTDYE

SEQ ID NO: 58 - protein, 8 aa, synthetic construct
  source 1..8: note = S43_HCDR2_IMGT
IDPAFGGT

SEQ ID NO: 59 - protein, 7 aa, synthetic construct
  source 1..7: note = S43_HCDR3_IMGT
ARPYLGY

SEQ ID NO: 60 - protein, 8 aa, synthetic construct
  source 1..8: note = 1-5_HCDR1_IMGT
GYTFTDYE

SEQ ID NO: 61 - protein, 8 aa, synthetic construct
  source 1..8: note = 1-5_HCDR2_IMGT
IDPETGGT

SEQ ID NO: 62 - protein, 7 aa, synthetic construct
  source 1..7: note = 1-5_HCDR3_IMGT
ARPYLGY

SEQ ID NO: 63 - protein, 8 aa, synthetic construct
  source 1..8: note = 2-1_HCDR1_IMGT
GYTFTDYE

SEQ ID NO: 64 - protein, 8 aa, synthetic construct
  source 1..8: note = 2-1_HCDR2_IMGT
IDPETGGT

SEQ ID NO: 65 - protein, 7 aa, synthetic construct
  source 1..7: note = 2-1_HCDR3_IMGT
ARPYLGY

SEQ ID NO: 66 - protein, 8 aa, synthetic construct
  source 1..8: note = E01_HCDR1_IMGT
GYTFTDYE

SEQ ID NO: 67 - protein, 8 aa, synthetic construct
  source 1..8: note = E01_HCDR2_IMGT
IDPETGGT

SEQ ID NO: 68 - protein, 7 aa, synthetic construct
  source 1..7: note = E01_HCDR3_IMGT
TRPYLGY

SEQ ID NO: 69 - protein, 11 aa, synthetic construct
  source 1..11: note = E01_LCDR1_IMGT
QSLVHRNGNTY

SEQ ID NO: 70 - skipped

SEQ ID NO: 71 - protein, 9 aa, synthetic construct
  source 1..9: note = E01_LCDR3_IMGT
FQGSHIPLT